European Patent Application EP 4 378 960 A1, published June 5, 2024. Title: ANTIGEN TARGETING, ANTI-CD16A, AND IMMUNE EFFECTOR CELL ACTIVATING TRIFUNCTIONAL FUSION PROTEIN, AND APPLICATION THEREOF. Applicant: QURE BIOTECHNOLOGY (SHANGHAI) CO., LTD. The sequence listing filed with the application follows.

SEQUENCE LISTING (54 sequences)

SEQ ID NO: 1 - protein, 257 aa, synthetic construct
MDMRVPAQLLGLLLLWFPGSRCSYVLTQPSSVSVAPGQTATISCGGHNIGSKNVHWYQQRPGQSPVLVIYQDNKRPSGIPERFSGSNSGNTATLTISGTQAMDEADYYCQVWDNYSVLFGGGTKLTVLGGGGSGGGGSGGGGSNWVNVISDLKKIEDLIQSMHIDATLYTESDVHPSCKVTAMKCFLLELQVISCESGDASIHDTVENLIILANNSLSSNGNVTESGCKECEELEEKNIKEFLQSFVHIVQMFINTS

SEQ ID NO: 2 - protein, 456 aa, synthetic construct
MEFGLSWLFLVAILKGVQCQVQLVQSGAEVKKPGESLKVSCKASGYTFTSYYMHWVRQAPGQGLEWMGIINPSGGSTSYAQKFQGRVTMTRDTSTSTVYMELSSLRSEDTAVYYCARGSAYYYDFADYWGQGTLVTVSSGGGGSGGGGSGGGGSITCPPPMSVEHADIWVKSYSLYSRERYICNSGFKRKAGTCSLTECVLNKATNVAHWTTPSLKCIRGGGGSEPKSSDKTHTCPPCPAPELLGGPSVFLFPPKPKDTLMISRTPEVTCVVVDVSHEDPEVKFNWYVDGVEVHNAKTKPREEQYNSTYRVVSVLTVLHQDWLNGKEYKCKVSNKALPAPIEKTISKAKGQPREPQVYTLPPSRDELTKNQVSLWCLVKGFYPSDIAVEWESNGQPENNYKTTPPVLDSDGSFFLYSKLTVDKSRWQQGNVFSCSVMHEALHNHYTQKSLSLSPGK

SEQ ID NO: 3 - protein, 242 aa, synthetic construct
MDMRVPAQLLGLLLLWFPGSRCDIVMTQSPDSLTVSLGERTTINCKSSQSVLDSSTNKNSLAWYQQKPGQPPKLLLSWASTRESGIPDRFSGSGSGTDFTLTIDSPQPEDSATYYCQQSAHFPITFGQGTRLEIKRTVAAPSVFIFPPSDEQLKSGTASVVCLLNNFYPREAKVQWKVDNALQSGNSQESVTEQDSKDSTYSLSSTLTLSKADYEKHKVYACEVTHQGLSSPVTKSFNRGEC

SEQ ID NO: 4 - protein, 471 aa, synthetic construct
MEFGLSWLFLVAILKGVQCQVQLVQSGAEVKKPGESVKVSCKASGYTFTNYGMNWVKQAPGQGLEWMGWINTYTGEPTYADKFQGRVTMTTDTSTSTAYMEIRNLGGDDTAVYYCARWSWSDGYYVYFDYWGQGTSVTVSSASTKGPSVFPLAPSSKSTSGGTAALGCLVKDYFPEPVTVSWNSGALTSGVHTFPAVLQSSGLYSLSSVVTVPSSSLGTQTYICNVNHKPSNTKVDKKVEPKSCDKTHTCPPCPAPELLGGPSVFLFPPKPKDTLMISRTPEVTCVVVDVSHEDPEVKFNWYVDGVEVHNAKTKPREEQYNSTYRVVSVLTVLHQDWLNGKEYKCKVSNKALPAPIEKTISKAKGQPREPQVYTLPPSREEMTKNQVSLSCAVKGFYPSDIAVEWESNGQPENNYKTTPPVLDSDGSFFLVSKLTVDKSRWQQGNVFSCSVMHEALHNRYTQKSLSLSPGK

SEQ ID NO: 5 - protein, 456 aa, synthetic construct
MEFGLSWLFLVAILKGVQCQVQLVQSGAEVKKPGESLKVSCKASGYTFTSYYMHWVRQAPGQGLEWMGIINPSGGSTSYAQKFQGRVTMTRDTSTSTVYMELSSLRSEDTAVYYCARGSAYYYDFADYWGQGTLVTVSSGGGGSGGGGSGGGGSITCPPPMSVEHADIWVKSYSLYSRERYICNSGFKRKAGTCSLTECVLNKATNVAHWTTPSLKCIRGGGGSEPKSSDKTHTCPPCPAPEAAGGPSVFLFPPKPKDTLMISRTPEVTCVVVDVSHEDPEVKFNWYVDGVEVHNAKTKPREEQYNSTYRVVSVLTVLHQDWLNGKEYKCKVSNKALPAPIEKTISKAKGQPREPQVYTLPPSRDELTKNQVSLWCLVKGFYPSDIAVEWESNGQPENNYKTTPPVLDSDGSFFLYSKLTVDKSRWQQGNVFSCSVMHEALHNHYTQKSLSLSPGK

SEQ ID NO: 6 - protein, 471 aa, synthetic construct
MEFGLSWLFLVAILKGVQCQVQLVQSGAEVKKPGESVKVSCKASGYTFTNYGMNWVKQAPGQGLEWMGWINTYTGEPTYADKFQGRVTMTTDTSTSTAYMEIRNLGGDDTAVYYCARWSWSDGYYVYFDYWGQGTSVTVSSASTKGPSVFPLAPSSKSTSGGTAALGCLVKDYFPEPVTVSWNSGALTSGVHTFPAVLQSSGLYSLSSVVTVPSSSLGTQTYICNVNHKPSNTKVDKKVEPKSCDKTHTCPPCPAPEAAGGPSVFLFPPKPKDTLMISRTPEVTCVVVDVSHEDPEVKFNWYVDGVEVHNAKTKPREEQYNSTYRVVSVLTVLHQDWLNGKEYKCKVSNKALPAPIEKTISKAKGQPREPQVYTLPPSREEMTKNQVSLSCAVKGFYPSDIAVEWESNGQPENNYKTTPPVLDSDGSFFLVSKLTVDKSRWQQGNVFSCSVMHEALHNRYTQKSLSLSPGK

SEQ ID NO: 7 - protein, 213 aa, synthetic construct
SYVLTQPSSVSVAPGQTATISCGGHNIGSKNVHWYQQRPGQSPVLVIYQDNKRPSGIPERFSGSNSGNTATLTISGTQAMDEADYYCQVWDNYSVLFGGGTKLTVLRTVAAPSVFIFPPSDEQLKSGTASVVCLLNNFYPREAKVQWKVDNALQSGNSQESVTEQDSKDSTYSLSSTLTLSKADYEKHKVYACEVTHQGLSSPVTKSFNRGEC

SEQ ID NO: 8 - protein, 478 aa, synthetic construct
MEFGLSWLFLVAILKGVQCQVQLVQSGAEVKKPGESLKVSCKASGYTFTSYYMHWVRQAPGQGLEWMGIINPSGGSTSYAQKFQGRVTMTRDTSTSTVYMELSSLRSEDTAVYYCARGSAYYYDFADYWGQGTLVTVSSASTKGPSVFPLAPSSKSTSGGTAALGCLVKDYFPEPVTVSWNSGALTSGVHTFPAVLQSSGLYSLSSVVTVPSSSLGTQTYICNVNHKPSNTKVDKKVEPKSCDKTHTCPPCPAPEAAGGPSVFLFPPKPKDTLMISRTPEVTCVVVDVSHEDPEVKFNWYVDGVEVHNAKTKPREEQYNSTYRVVSVLTVLHQDWLNGKEYKCKVSNKALPAPIEKTISKAKGQPREPQVYTLPPSREEMTKNQVSLSCAVKGFYPSDIAVEWESNGQPENNYKTTPPVLDSDGSFFLVSKLTVDKSRWQQGNVFSCSVMHEALHNRYTQKSLSLSPGKGGSHHHHHH

SEQ ID NO: 9 - protein, 469 aa, synthetic construct
MEFGLSWLFLVAILKGVQCQVQLVQSGAEVKKPGESVKVSCKASGYTFTNYGMNWVKQAPGQGLEWMGWINTYTGEPTYADKFQGRVTMTTDTSTSTAYMEIRNLGGDDTAVYYCARWSWSDGYYVYFDYWGQGTSVTVSSGGGGSGGGGSGGGGSITCPPPMSVEHADIWVKSYSLYSRERYICNSGFKRKAGTCSLTECVLNKATNVAHWTTPSLKCIRGGGGSEPKSSDKTHTCPPCPAPEAAGGPSVFLFPPKPKDTLMISRTPEVTCVVVDVSHEDPEVKFNWYVDGVEVHNAKTKPREEQYNSTYRVVSVLTVLHQDWLNGKEYKCKVSNKALPAPIEKTISKAKGQPREPQVYTLPPSRDELTKNQVSLWCLVKGFYPSDIAVEWESNGQPENNYKTTPPVLDSDGSFFLYSKLTVDKSRWQQGNVFSCSVMHEALHNHYTQKSLSLSPGKGGSDYKDDDDK

SEQ ID NO: 10 - protein, 242 aa, synthetic construct
DIVMTQSPDSLTVSLGERTTINCKSSQSVLDSSTNKNSLAWYQQKPGQPPKLLLSWASTRESGIPDRFSGSGSGTDFTLTIDSPQPEDSATYYCQQSAHFPITFGQGTRLEIKGGGGSGGGGSGGGGSNWVNVISDLKKIEDLIQSMHIDATLYTESDVHPSCKVTAMKCFLLELQVISCESGDASIHDTVENLIILANNSLSSNGNVTESGCKECEELEEKNIKEFLQSFVHIVQMFINTS

SEQ ID NO: 11 - protein, 236 aa, synthetic construct
MDMRVPAQLLGLLLLWFPGSRCEIVLTQSPATLSLSPGERATLSCRASQSVSSYLAWYQQKPGQAPRLLIYDASNRATGIPARFSGSGSGTDFTLTISSLEPEDFAVYYCQQRSNWPPTFGQGTKVEIKRTVAAPSVFIFPPSDEQLKSGTASVVCLLNNFYPREAKVQWKVDNALQSGNSQESVTEQDSKDSTYSLSSTLTLSKADYEKHKVYACEVTHQGLSSPVTKSFNRGEC

SEQ ID NO: 12 - protein, 471 aa, synthetic construct
MEFGLSWLFLVAILKGVQCEVQLLESGGGLVQPGGSLRLSCAVSGFTFNSFAMSWVRQAPGKGLEWVSAISGSGGGTYYADSVKGRFTISRDNSKNTLYLQMNSLRAEDTAVYFCAKDKILWFGEPVFDYWGQGTLVTVSSASTKGPSVFPLAPSSKSTSGGTAALGCLVKDYFPEPVTVSWNSGALTSGVHTFPAVLQSSGLYSLSSVVTVPSSSLGTQTYICNVNHKPSNTKVDKKVEPKSCDKTHTCPPCPAPELLGGPSVFLFPPKPKDTLMISRTPEVTCVVVDVSHEDPEVKFNWYVDGVEVHNAKTKPREEQYNSTYRVVSVLTVLHQDWLNGKEYKCKVSNKALPAPIEKTISKAKGQPREPQVYTLPPSREEMTKNQVSLSCAVKGFYPSDIAVEWESNGQPENNYKTTPPVLDSDGSFFLVSKLTVDKSRWQQGNVFSCSVMHEALHNRYTQKSLSLSPGK

SEQ ID NO: 13 - protein, 236 aa, synthetic construct
MDMRVPAQLLGLLLLWFPGSRCDIQMTQSPSSLSASVGDRVTITCKASQDVGIAVAWYQQKPGKVPKLLIYWASTRHTGVPDRFSGSGSGTDFTLTISSLQPEDVATYYCQQYSSYPYTFGQGTKVEIKRTVAAPSVFIFPPSDEQLKSGTASVVCLLNNFYPREAKVQWKVDNALQSGNSQESVTEQDSKDSTYSLSSTLTLSKADYEKHKVYACEVTHQGLSSPVTKSFNRGEC

SEQ ID NO: 14 - protein, 477 aa, synthetic construct
MEFGLSWLFLVAILKGVQCEVQLVESGGGLVQPGGSLRLSCAASGFDFSRYWMSWVRQAPGKGLEWIGEINPDSSTINYAPSLKDKFIISRDNAKNSLYLQMNSLRAEDTAVYYCARPDGNYWYFDVWGQGTLVTVSSASTKGPSVFPLAPSSKSTSGGTAALGCLVKDYFPEPVTVSWNSGALTSGVHTFPAVLQSSGLYSLSSVVTVPSSSLGTQTYICNVNHKPSNTKVDKKVEPKSCDKTHTCPPCPAPELLGGPSVFLFPPKPKDTLMISRTPEVTCVVVDVSHEDPEVKFNWYVDGVEVHNAKTKPREEQYNSTYRVVSVLTVLHQDWLNGKEYKCKVSNKALPAPIEKTISKAKGQPREPQVYTLPPSREEMTKNQVSLSCAVKGFYPSDIAVEWESNGQPENNYKTTPPVLDSDGSFFLVSKLTVDKSRWQQGNVFSCSVMHEALHNRYTQKSLSLSPGKGGSHHHHHH

SEQ ID NO: 15 - protein, 471 aa, synthetic construct
MEFGLSWLFLVAILKGVQCEVQLLESGGGLVQPGGSLRLSCAVSGFTFNSFAMSWVRQAPGKGLEWVSAISGSGGGTYYADSVKGRFTISRDNSKNTLYLQMNSLRAEDTAVYFCAKDKILWFGEPVFDYWGQGTLVTVSSASTKGPSVFPLAPSSKSTSGGTAALGCLVKDYFPEPVTVSWNSGALTSGVHTFPAVLQSSGLYSLSSVVTVPSSSLGTQTYICNVNHKPSNTKVDKKVEPKSCDKTHTCPPCPAPEAAGGPSVFLFPPKPKDTLMISRTPEVTCVVVDVSHEDPEVKFNWYVDGVEVHNAKTKPREEQYNSTYRVVSVLTVLHQDWLNGKEYKCKVSNKALPAPIEKTISKAKGQPREPQVYTLPPSREEMTKNQVSLSCAVKGFYPSDIAVEWESNGQPENNYKTTPPVLDSDGSFFLVSKLTVDKSRWQQGNVFSCSVMHEALHNRYTQKSLSLSPGK

SEQ ID NO: 16 - protein, 477 aa, synthetic construct
MEFGLSWLFLVAILKGVQCEVQLVESGGGLVQPGGSLRLSCAASGFDFSRYWMSWVRQAPGKGLEWIGEINPDSSTINYAPSLKDKFIISRDNAKNSLYLQMNSLRAEDTAVYYCARPDGNYWYFDVWGQGTLVTVSSASTKGPSVFPLAPSSKSTSGGTAALGCLVKDYFPEPVTVSWNSGALTSGVHTFPAVLQSSGLYSLSSVVTVPSSSLGTQTYICNVNHKPSNTKVDKKVEPKSCDKTHTCPPCPAPEAAGGPSVFLFPPKPKDTLMISRTPEVTCVVVDVSHEDPEVKFNWYVDGVEVHNAKTKPREEQYNSTYRVVSVLTVLHQDWLNGKEYKCKVSNKALPAPIEKTISKAKGQPREPQVYTLPPSREEMTKNQVSLSCAVKGFYPSDIAVEWESNGQPENNYKTTPPVLDSDGSFFLVSKLTVDKSRWQQGNVFSCSVMHEALHNRYTQKSLSLSPGKGGSHHHHHH

SEQ ID NO: 17 - protein, 242 aa, synthetic construct; identical to SEQ ID NO: 3

SEQ ID NO: 18 - protein, 471 aa, synthetic construct
MEFGLSWLFLVAILKGVQCQVQLVQSGAEVKKPGESVKVSCKASGYTFTNYGMNWVKQAPGQGLEWMGWINTYTGEPTYADKFQGRVTMTTDTSTSTAYMEIRNLGGDDTAVYYCARWSWSDGYYVYFDYWGQGTSVTVSSASTKGPSVFPLAPSSKSTSGGTAALGCLVKDYFPEPVTVSWNSGALTSGVHTFPAVLQSSGLYSLSSVVTVPSSSLGTQTYICNVNHKPSNTKVDKKVEPKSCDKTHTCPPCPAPELLGGPSVFLFPPKPKDTLMISRTPEVTCVVVDVSHEDPEVKFNWYVDGVEVHNAKTKPREEQYNSTYRVVSVLTVLHQDWLNGKEYKCKVSNKALPAPIEKTISKAKGQPREPQVYTLPPSRDELTKNQVSLTCLVKGFYPSDIAVEWESNGQPENNYKTTPPVLDSDGSFFLYSKLTVDKSRWQQGNVFSCSVMHEALHNHYTQKSLSLSPGK

SEQ ID NO: 19 - protein, 468 aa, synthetic construct
MEFGLSWLFLVAILKGVQCEVQLVESGGGLVQPGGSLRLSCAASGFDFSRYWMSWVRQAPGKGLEWIGEINPDSSTINYAPSLKDKFIISRDNAKNSLYLQMNSLRAEDTAVYYCARPDGNYWYFDVWGQGTLVTVSSASTKGPSVFPLAPSSKSTSGGTAALGCLVKDYFPEPVTVSWNSGALTSGVHTFPAVLQSSGLYSLSSVVTVPSSSLGTQTYICNVNHKPSNTKVDKKVEPKSCDKTHTCPPCPAPELLGGPSVFLFPPKPKDTLMISRTPEVTCVVVDVSHEDPEVKFNWYVDGVEVHNAKTKPREEQYNSTYRVVSVLTVLHQDWLNGKEYKCKVSNKALPAPIEKTISKAKGQPREPQVYTLPPSRDELTKNQVSLTCLVKGFYPSDIAVEWESNGQPENNYKTTPPVLDSDGSFFLYSKLTVDKSRWQQGNVFSCSVMHEALHNHYTQKSLSLSPGK

SEQ ID NO: 20 - protein, 236 aa, synthetic construct; identical to SEQ ID NO: 13

SEQ ID NO: 21 - protein, 471 aa, synthetic construct
MEFGLSWLFLVAILKGVQCEVQLLESGGGLVQPGGSLRLSCAVSGFTFNSFAMSWVRQAPGKGLEWVSAISGSGGGTYYADSVKGRFTISRDNSKNTLYLQMNSLRAEDTAVYFCAKDKILWFGEPVFDYWGQGTLVTVSSASTKGPSVFPLAPSSKSTSGGTAALGCLVKDYFPEPVTVSWNSGALTSGVHTFPAVLQSSGLYSLSSVVTVPSSSLGTQTYICNVNHKPSNTKVDKKVEPKSCDKTHTCPPCPAPELLGGPSVFLFPPKPKDTLMISRTPEVTCVVVDVSHEDPEVKFNWYVDGVEVHNAKTKPREEQYNSTYRVVSVLTVLHQDWLNGKEYKCKVSNKALPAPIEKTISKAKGQPREPQVYTLPPSRDELTKNQVSLTCLVKGFYPSDIAVEWESNGQPENNYKTTPPVLDSDGSFFLYSKLTVDKSRWQQGNVFSCSVMHEALHNHYTQKSLSLSPGK

SEQ ID NO: 22 - protein, 236 aa, synthetic construct; identical to SEQ ID NO: 11

SEQ ID NO: 23 - protein, 469 aa, synthetic construct
MEFGLSWLFLVAILKGVQCQVQLVQSGAEVKKPGESLKVSCKASGYTFTSYYMHWVRQAPGQGLEWMGIINPSGGSTSYAQKFQGRVTMTRDTSTSTVYMELSSLRSEDTAVYYCARGSAYYYDFADYWGQGTLVTVSSASTKGPSVFPLAPSSKSTSGGTAALGCLVKDYFPEPVTVSWNSGALTSGVHTFPAVLQSSGLYSLSSVVTVPSSSLGTQTYICNVNHKPSNTKVDKKVEPKSCDKTHTCPPCPAPEAAGGPSVFLFPPKPKDTLMISRTPEVTCVVVDVSHEDPEVKFNWYVDGVEVHNAKTKPREEQYNSTYRVVSVLTVLHQDWLNGKEYKCKVSNKALPAPIEKTISKAKGQPREPQVYTLPPSRDELTKNQVSLTCLVKGFYPSDIAVEWESNGQPENNYKTTPPVLDSDGSFFLYSKLTVDKSRWQQGNVFSCSVMHEALHNHYTQKSLSLSPGK

SEQ ID NO: 24 - protein, 235 aa, synthetic construct
MDMRVPAQLLGLLLLWFPGSRCSYVLTQPSSVSVAPGQTATISCGGHNIGSKNVHWYQQRPGQSPVLVIYQDNKRPSGIPERFSGSNSGNTATLTISGTQAMDEADYYCQVWDNYSVLFGGGTKLTVLRTVAAPSVFIFPPSDEQLKSGTASVVCLLNNFYPREAKVQWKVDNALQSGNSQESVTEQDSKDSTYSLSSTLTLSKADYEKHKVYACEVTHQGLSSPVTKSFNRGEC

SEQ ID NO: 25 - protein, 508 aa, synthetic construct
MEFGLSWLFLVAILKGVQCQVQLVQSGAEVKKPGESLKVSCKASGYTFTSYYMHWVRQAPGQGLEWMGIINPSGGSTSYAQKFQGRVTMTRDTSTSTVYMELSSLRSEDTAVYYCARGSAYYYDFADYWGQGTLVTVSSGGGGSGGGGSGGGGSSYVLTQPSSVSVAPGQTATISCGGHNIGSKNVHWYQQRPGQSPVLVIYQDNKRPSGIPERFSGSNSGNTATLTISGTQAMDEADYYCQVWDNYSVLFGGGTKLTVLGGGGSEPKSSDKTHTCPPCPAPELLGGPSVFLFPPKPKDTLMISRTPEVTCVVVDVSHEDPEVKFNWYVDGVEVHNAKTKPREEQYNSTYRVVSVLTVLHQDWLNGKEYKCKVSNKALPAPIEKTISKAKGQPREPQVYTLPPSRDELTKNQVSLWCLVKGFYPSDIAVEWESNGQPENNYKTTPPVLDSDGSFFLYSKLTVDKSRWQQGNVFSCSVMHEALHNHYTQKSLSLSPGKGGSDYKDDDDK

SEQ ID NO: 26 - protein, 480 aa, synthetic construct
MEFGLSWLFLVAILKGVQCQVQLVQSGAEVKKPGESVKVSCKASGYTFTNYGMNWVKQAPGQGLEWMGWINTYTGEPTYADKFQGRVTMTTDTSTSTAYMEIRNLGGDDTAVYYCARWSWSDGYYVYFDYWGQGTSVTVSSASTKGPSVFPLAPSSKSTSGGTAALGCLVKDYFPEPVTVSWNSGALTSGVHTFPAVLQSSGLYSLSSVVTVPSSSLGTQTYICNVNHKPSNTKVDKKVEPKSCDKTHTCPPCPAPELLGGPSVFLFPPKPKDTLMISRTPEVTCVVVDVSHEDPEVKFNWYVDGVEVHNAKTKPREEQYNSTYRVVSVLTVLHQDWLNGKEYKCKVSNKALPAPIEKTISKAKGQPREPQVYTLPPSREEMTKNQVSLSCAVKGFYPSDIAVEWESNGQPENNYKTTPPVLDSDGSFFLVSKLTVDKSRWQQGNVFSCSVMHEALHNRYTQKSLSLSPGKGGSHHHHHH

SEQ ID NO: 27 - protein, 242 aa, synthetic construct; identical to SEQ ID NO: 3

SEQ ID NO: 28 - protein, 508 aa, synthetic construct; identical to SEQ ID NO: 25

SEQ ID NO: 29 - protein, 480 aa, synthetic construct; identical to SEQ ID NO: 26

SEQ ID NO: 30 - protein, 242 aa, synthetic construct; identical to SEQ ID NO: 3

SEQ ID NO: 31 - protein, 641 aa, synthetic construct
MEFGLSWLFLVAILKGVQCEVQLVESGGGVVRPGGSLRLSCAASGFTFDDYGMSWVRQAPGKGLEWVSGINWNGGSTGYADSVKGRFTISRDNAKNSLYLQMNSLRAEDTAVYYCARGRSLLFDYWGQGTLVTVSRGGGGSGGGGSGGGGSSELTQDPAVSVALGQTVRITCQGDSLRSYYASWYQQKPGQAPVLVIYGKNNRPSGIPDRFSGSSSGNTASLTITGAQAEDEADYYCNSRDSSGNHVVFGGGTKLTVLPSGQAGAAASESLFVSNHAYNWVNVISDLKKIEDLIQSMHIDATLYTESDVHPSCKVTAMKCFLLELQVISLESGDASIHDTVENLIILANDSLSSNGNVTESGCKECEELEEKNIKEFLQSFVHIVQMFINTSEASGGPEQVQLVQSGAEVKKPGSSVKVSCKASGYTFTDYNMHWVRQAPGQGLEWIGYIYPYNGGTGYNQKFKSKATITADESTNTAYMELSSLRSEDTAVYYCARGRPAMDYWGQGTLVTVSSGGGGSGGGGSGGGGSDIQMTQSPSSLSASVGDRVTITCRASESVDNYGISFMNWFQQKPGKAPKLLIYAASNQGSGVPSRFSGSGSGTDFTLTISSLQPDDFATYYCQQSKEVPWTFGQGTKVEIK

SEQ ID NO: 32 - protein, 133 aa, synthetic construct
MEFGLSWLFLVAILKGVQCNWVNVISDLKKIEDLIQSMHIDATLYTESDVHPSCKVTAMKCFLLELQVISCESGDASIHDTVENLIILANNSLSSNGNVTESGCKECEELEEKNIKEFLQSFVHIVQMFINTS

SEQ ID NO: 33 - protein, 344 aa, synthetic construct
MEFGLSWLFLVAILKGVQCITCPPPMSVEHADIWVKSYSLYSRERYICNSGFKRKAGTCSLTECVLNKATNVAHWTTPSLKCIRDPALVHQRSGGSGGGGSGGGSGGGGSLQEPKSSDKTHTCPPCPAPELLGGPSVFLFPPKPKDTLMISRTPEVTCVVVDVSHEDPEVKFNWYVDGVEVHNAKTKPREEQYNSTYRVVSVLTVLHQDWLNGKEYKCKVSNKALPAPIEKTISKAKGQPREPQVYTLPPSRDELTKNQVSLTCLVKGFYPSDIAVEWESNGQPENNYKTTPPVLDSDGSFFLYSKLTVDKSRWQQGNVFSCSVMHEALHNHYTQKSLSLSPGK

SEQ ID NO: 34 - protein, 508 aa, synthetic construct; identical to SEQ ID NO: 25

SEQ ID NO: 35 - protein, 477 aa, synthetic construct; identical to SEQ ID NO: 16

SEQ ID NO: 36 - protein, 508 aa, synthetic construct; identical to SEQ ID NO: 25

SEQ ID NO: 37 - protein, 480 aa, synthetic construct
MEFGLSWLFLVAILKGVQCEVQLLESGGGLVQPGGSLRLSCAVSGFTFNSFAMSWVRQAPGKGLEWVSAISGSGGGTYYADSVKGRFTISRDNSKNTLYLQMNSLRAEDTAVYFCAKDKILWFGEPVFDYWGQGTLVTVSSASTKGPSVFPLAPSSKSTSGGTAALGCLVKDYFPEPVTVSWNSGALTSGVHTFPAVLQSSGLYSLSSVVTVPSSSLGTQTYICNVNHKPSNTKVDKKVEPKSCDKTHTCPPCPAPEAAGGPSVFLFPPKPKDTLMISRTPEVTCVVVDVSHEDPEVKFNWYVDGVEVHNAKTKPREEQYNSTYRVVSVLTVLHQDWLNGKEYKCKVSNKALPAPIEKTISKAKGQPREPQVYTLPPSREEMTKNQVSLSCAVKGFYPSDIAVEWESNGQPENNYKTTPPVLDSDGSFFLVSKLTVDKSRWQQGNVFSCSVMHEALHNRYTQKSLSLSPGKGGSHHHHHH

SEQ ID NO: 38 - protein, 106 aa, synthetic construct
SYVLTQPSSVSVAPGQTATISCGGHNIGSKNVHWYQQRPGQSPVLVIYQDNKRPSGIPERFSGSNSGNTATLTISGTQAMDEADYYCQVWDNYSVLFGGGTKLTVL

SEQ ID NO: 39 - protein, 120 aa, synthetic construct
QVQLVQSGAEVKKPGESLKVSCKASGYTFTSYYMHWVRQAPGQGLEWMGIINPSGGSTSYAQKFQGRVTMTRDTSTSTVYMELSSLRSEDTAVYYCARGSAYYYDFADYWGQGTLVTVSS

SEQ ID NO: 40 - protein, 107 aa, synthetic construct [sequence omitted]

SEQ ID NO: 41 - protein, 122 aa, synthetic construct [sequence omitted]

SEQ ID NO: 42 - protein, 107 aa, synthetic construct
DIQMTQSPSSLSASVGDRVTITCKASQDVGIAVAWYQQKPGKVPKLLIYWASTRHTGVPDRFSGSGSGTDFTLTISSLQPEDVATYYCQQYSSYPYTFGQGTKVEIK

SEQ ID NO: 43 - protein, 119 aa, synthetic construct
EVQLVESGGGLVQPGGSLRLSCAASGFDFSRYWMSWVRQAPGKGLEWIGEINPDSSTINYAPSLKDKFIISRDNAKNSLYLQMNSLRAEDTAVYYCARPDGNYWYFDVWGQGTLVTVSS

SEQ ID NO: 44 - protein, 113 aa, synthetic construct
DIVMTQSPDSLTVSLGERTTINCKSSQSVLDSSTNKNSLAWYQQKPGQPPKLLLSWASTRESGIPDRFSGSGSGTDFTLTIDSPQPEDSATYYCQQSAHFPITFGQGTRLEIK

SEQ ID NO: 45 - protein, 122 aa, synthetic construct
QVQLVQSGAEVKKPGESVKVSCKASGYTFTNYGMNWVKQAPGQGLEWMGWINTYTGEPTYADKFQGRVTMTTDTSTSTAYMEIRNLGGDDTAVYYCARWSWSDGYYVYFDYWGQGTSVTVSS

SEQ ID NO: 46 - protein, 114 aa, synthetic construct
NWVNVISDLKKIEDLIQSMHIDATLYTESDVHPSCKVTAMKCFLLELQVISLESGDASIHDTVENLIILANNSLSSNGNVTESGCKECEELEEKNIKEFLQSFVHIVQMFINTS

SEQ ID NO: 47 - protein, 114 aa, synthetic construct
NWVNVISDLKKIEDLIQSMHIDATLYTESDVHPSCKVTAMKCFLLELQVISCESGDASIHDTVENLIILANNSLSSNGNVTESGCKECEELEEKNIKEFLQSFVHIVQMFINTS

SEQ ID NO: 48 - protein, 175 aa, synthetic construct
ITCPPPMSVEHADIWVKSYSLYSRERYICNSGFKRKAGTSSLTECVLNKATNVAHWTTPSLKCIRDPALVHQRPAPPSTVTTAGVTPQPESLSPSGKEPAASSPSSNNTAATTAAIVPGSQLMPSKSPSTGTTEISSHESSHGTPSQTTAKNWELTASASHQPPGVYPQGHSDTT

SEQ ID NO: 49 - protein, 65 aa, synthetic construct
ITCPPPMSVEHADIWVKSYSLYSRERYICNSGFKRKAGTSSLTECVLNKATNVAHWTTPSLKCIR

SEQ ID NO: 50 - protein, 73 aa, synthetic construct
ITCPPPMSVEHADIWVKSYSLYSRERYICNSGFKRKAGTSSLTECVLNKATNVAHWTTPSLKCIRDPALVHQR

SEQ ID NO: 51 - protein, 77 aa, synthetic construct
ITCPPPMSVEHADIWVKSYSLYSRERYICNSGFKRKAGTSSLTECVLNKATNVAHWTTPSLKCIRDPALVHQRPAPP

SEQ ID NO: 52 - protein, 86 aa, synthetic construct
ITCPPPMSVEHADIWVKSYSLYSRERYICNSGFKRKAGTSSLTECVLNKATNVAHWTTPSLKCIRDPALVHQRPAPPSTVTTAGVT

SEQ ID NO: 53 - protein, 102 aa, synthetic construct
ITCPPPMSVEHADIWVKSYSLYSRERYICNSGFKRKAGTSSLTECVLNKATNVAHWTTPSLKCIRDPALVHQRPAPPSTVTTAGVTPQPESLSPSGKEPAAS

SEQ ID NO: 54 - protein, 65 aa, synthetic construct
ITCPPPMSVEHADIWVKSYSLYSRERYICNSGFKRKAGTCSLTECVLNKATNVAHWTTPSLKCIR